European Patent Specification EP 3 617 308 B1, published October 25, 2023. Title: PHI29 DNA POLYMERASE MUTANT WITH INCREASED THERMOSTABILITY. Applicant: MGI TECH CO., LTD. The sequence listing filed with the application follows.

SEQUENCE LISTING (2 sequences)

SEQ ID NO: 1 - DNA, 1728 bp, Artificial sequence
  Nucleotide sequence encoding wild-type phi29 DNA polymerase
atgaagcatatgccgcgcaaaatgtatagctgcgactttgaaaccaccaccaaagtggaagattgccgcgtttgggcgtatggctatatgaacatcgaagaccacagcgaatacaaaattggcaacagcctggatgaatttatggcgtgggtgctgaaagttcaggcggatctgtattttcacaacctgaaatttgacggcgcgttcattattaactggctggaacgcaacggctttaaatggagcgcggatggcttaccgaacacctataacaccattattagccgcatgggccagtggtatatgattgatatctgcctgggctataaaggcaaacgcaagattcataccgtgatctatgatagcctgaagaaactgccgtttccggtgaaaaaaatcgcgaaggactttaaactgaccgtgctgaaaggcgatattgactaccataaagaacgcccggtgggctataaaattaccccggaggaatatgcgtacatcaagaacgacatccagattattgcggaagcgctgctgattcagtttaaacagggcctggatcgtatgaccgcgggtagcgatagcctgaaaggctttaaggacattatcaccaccaagaagttcaagaaagtgtttccgaccctgagcctgggcctggataaagaagtgcgctatgcgtatcgcggtggctttacctggctgaacgatcgctttaaggaaaaggaaattggcgaaggcatggtgtttgatgtgaacagcctgtatccggcgcagatgtatagccgcctgctgccgtatggtgaaccgattgtgtttgaaggcaagtatgtgtgggatgaagattatccgctgcacattcagcatattcgctgcgaattcgaactgaaggaaggctatattccgaccattcagattaaacgcagccgcttttataaaggcaacgagtacctgaaaagcagcggcggcgaaattgcggatctgtggctgagcaacgtggatctggaactgatgaaagaacactacgatctgtacaacgtggaatatatcagcggcctgaaatttaaagcgaccaccggcctgtttaaggactttatcgacaagtggacctacattaaaaccaccagcgaaggcgcgattaaacagctggcgaaactgatgctgaacagcctgtatggcaaatttgcgagcaacccggatgttaccggcaaagtgccgtatctgaaagaaaacggcgcgctgggctttcgtttaggcgaagaggaaaccaaagatccggtgtataccccgatgggcgtgtttattaccgcgtgggcgcgctataccaccattaccgcggcgcaggcgtgttatgatcgcattatctattgcgataccgatagcattcatctgaccggcaccgaaattccggatgtgatcaaagatattgtggacccgaaaaaactgggctattgggcgcatgaaagcacctttaaacgcgcgaaatatctgcgccagaaaacctatatccaggacatctacatgaaagaggtggatggcaaactggttgaaggcagcccggatgattataccgatattaagttcagcgtgaaatgcgcgggcatgaccgataaaattaagaaggaagtgaccttcgagaactttaaagtgggctttagccgcaaaatgaaaccgaaaccggttcaggtgcctggcggtgttgttctggtggatgataccttcaccatcaagtga

SEQ ID NO: 2 - protein, 575 aa, Artificial sequence [sequence omitted]